European Patent Application EP 4 736 954 A2, published May 6, 2026. Title: BISPECIFIC BINDING PROTEINS AND USES THEREOF. Applicant: MedImmune, LLC. Application US 62/332,788, filed May 6, 2016. The sequence listing filed with the application follows.

SEQUENCE LISTING (97 sequences)

SEQ ID NO: 1 - protein, 711 aa, synthetic construct
  REGION 1..711: note = Description of Artificial Sequence: Syntheticpolypeptide
DIQMTQSPSSLSASVGDRVTITCRASQSINSYLDWYQQKPGKAPKLLIYAASSLQSGVPSRFSGSGSGTDFTLTISSLQPEDFATYYCQQYYSTPFTFGCGTKVEIKGGGGSGGGGSGGGGSGGGGSQVQLVESGGGVVQPGRSLRLSCAASGFTFSSYGMHWVRQAPGKCLEWVAVIWYDGSNKYYADSVKGRFTISRDNSKNTLYLQMNSLRAEDTAVYYCARDPRGATLYYYYYGMDVWGQGTTVTVSSGGGGSGGGGSEVQLVESGGGLVQPGGSLRLSCAASGFTFSDYGMHWVRQAPGKGLEWVAYISSGSYTIYSADSVKGRFTISRDNAKNSLYLQMNSLRAEDTAVYYCARRAPNSFYEYYFDYWGQGTTVTVSSASTKGPSVFPLAPCSRSTSESTAALGCLVKDYFPEPVTVSWNSGALTSGVHTFPAVLQSSGLYSLSSVVTVPSSSLGTKTYTCNVDHKPSNTKVDKRVESKYGPPCPPCPAPEFLGGPSVFLFPPKPKDTLMISRTPEVTCVVVDVSQEDPEVQFNWYVDGVEVHNAKTKPREEQFNSTYRVVSVLTVLHQDWLNGKEYKCKVSNKGLPSSIEKTISKAKGQPREPQVYTLPPSQEEMTKNQVSLTCLVKGFYPSDIAVEWESNGQPENNYKTTPPVLDSDGSFFLYSRLTVDKSRWQEGNVFSCSVMHEALHNHYTQKSLSLSLGK

SEQ ID NO: 2 - protein, 219 aa, synthetic construct
  REGION 1..219: note = Description of Artificial Sequence: Syntheticpolypeptide
QIVLTQSPATLSLSPGERATLSCSASSKHTNLYWSRHMYWYQQKPGQAPRLLIYLTSNRATGIPARFSGSGSGTDFTLTISSLEPEDFAVYYCQQWSSNPFTFGQGTKLEIKRTVAAPSVFIFPPSDEQLKSGTASVVCLLNNFYPREAKVQWKVDNALQSGNSQESVTEQDSKDSTYSLSSTLTLSKADYEKHKVYACEVTHQGLSSPVTKSFNRGEC

SEQ ID NO: 3 - protein, 711 aa, synthetic construct
  REGION 1..711: note = Description of Artificial Sequence: Syntheticpolypeptide
EVQLVESGGGLVQPGGSLRLSCAASGFTFSDYGMHWVRQAPGKGLEWVAYISSGSYTIYSADSVKGRFTISRDNAKNSLYLQMNSLRAEDTAVYYCARRAPNSFYEYYFDYWGQGTTVTVSSASTKGPSVFPLAPCSRSTSESTAALGCLVKDYFPEPVTVSWNSGALTSGVHTFPAVLQSSGLYSLSSVVTVPSSSLGTKTYTCNVDHKPSNTKVDKRVESKYGPPCPPCPAPEFLGGPSVFLFPPKPKDTLMISRTPEVTCVVVDVSQEDPEVQFNWYVDGVEVHNAKTKPREEQFNSTYRVVSVLTVLHQDWLNGKEYKCKVSNKGLPSSIEKTISKAKGQPREPQVYTLPPSQEEMTKNQVSLTCLVKGFYPSDIAVEWESNGQPENNYKTTPPVLDSDGSFFLYSRLTVDKSRWQEGNVFSCSVMHEALHNHYTQKSLSLSLGKGGGGSGGGGSDIQMTQSPSSLSASVGDRVTITCRASQSINSYLDWYQQKPGKAPKLLIYAASSLQSGVPSRFSGSGSGTDFTLTISSLQPEDFATYYCQQYYSTPFTFGCGTKVEIKGGGGSGGGGSGGGGSGGGGSQVQLVESGGGVVQPGRSLRLSCAASGFTFSSYGMHWVRQAPGKCLEWVAVIWYDGSNKYYADSVKGRFTISRDNSKNTLYLQMNSLRAEDTAVYYCARDPRGATLYYYYYGMDVWGQGTTVTVSS

SEQ ID NO: 4 - protein, 213 aa, synthetic construct
  REGION 1..213: note = Description of Artificial Sequence: Syntheticpolypeptide
DIQMTQSPSSLSASVGDRVTITCRASQSINSYLDWYQQKPGKAPKLLIYAASSLQSGVPSRFSGSGSGTDFTLTISSLQPEDFATYYCQQYYSTPFTFGPGTKVEIKGQPKAAPSVTLFPPCSEELQANKATLVCLISDFYPGAVTVAWKADSSPVKAGVETTTPSKQSNNKYAASSYLSLTPEQWKSHRSYSCQVTHEGSTVEKTVAPTEVS

SEQ ID NO: 5 - protein, 721 aa, synthetic construct
  REGION 1..721: note = Description of Artificial Sequence: Syntheticpolypeptide
EVQLVESGGGLVQPGGSLRLSCAASGFTFSDYGMHWVRQAPGKGLEWVAYISSGSYTIYSADSVKGRFTISRDNAKNSLYLQMNSLRAEDTAVYYCARRAPNSFYEYYFDYWGQGTTVTVSSASTKGPSVFPLAPCSRSTSESTAALGCLVKDYFPEPVTVSWNSGALTSGVHTFPAVLQSSGLYSLSSVVTVPSSSLGTKTYTCNVDHKPSNTKVDKRVESKYGPPCPPCPAPEFLGGPSVFLFPPKPKDTLMISRTPEVTCVVVDVSQEDPEVQFNWYVDGVEVHNAKTKPREEQFNSTYRVVSVLTVLHQDWLNGKEYKCKVSNKGLPSSIEKTISKAKGQPREPQVYTLPPSQEEMTKNQVSLTCLVKGFYPSDIAVEWESNGGGGSGGGGSDIQMTQSPSSLSASVGDRVTITCRASQSINSYLDWYQQKPGKAPKLLIYAASSLQSGVPSRFSGSGSGTDFTLTISSLQPEDFATYYCQQYYSTPFTFGCGTKVEIKGGGGSGGGGSGGGGSGGGGSQVQLVESGGGVVQPGRSLRLSCAASGFTFSSYGMHWVRQAPGKCLEWVAVIWYDGSNKYYADSVKGRFTISRDNSKNTLYLQMNSLRAEDTAVYYCARDPRGATLYYYYYGMDVWGQGTTVTVSSGGGGSGGGGSGQPENNYKTTPPVLDSDGSFFLYSRLTVDKSRWQEGNVFSCSVMHEALHNHYTQKSLSLSLGK

SEQ ID NO: 6 - protein, 219 aa, synthetic construct; identical to SEQ ID NO: 2
  REGION 1..219: note = Description of Artificial Sequence: Syntheticpolypeptide

SEQ ID NO: 7 - protein, 219 aa, synthetic construct; identical to SEQ ID NO: 2
  REGION 1..219: note = Description of Artificial Sequence: Syntheticpolypeptide

SEQ ID NO: 8 - DNA, 610 bp, synthetic construct
  misc_feature 1..610: note = Description of Artificial Sequence: Synthetic polynucleotide
  source 1..610: mol_type = other DNA
cgagagagccaccctgagctgctccgcctcctccaagcacaccaacctgtactggtcccggcacatgtactggtatcagcagaagcccggccaggcccctcggctgctgatctacctgacctctaaccgggccaccggcatccctgccagattctccggctctggctccggcaccgacttcaccctgaccatctccagcctggaacccgaggacttcgccgtgtactactgccagcagtggtcctccaaccccttcaccttcggccagggcaccaagctggaaatcaagcgtacggtggctgcaccatctgtcttcatcttcccgccatctgatgagcagttgaaatctggaactgcctctgttgtgtgcctgctgaataacttctatcccagagaggccaaagtacagtggaaggtggataacgccctccaatcgggtaactcccaggagagtgtcacagagcaggacagcaaggacagcacctacagcctcagcagcaccctgacgctgagcaaagcagactacgagaaacacaaagtctacgcctgcgaagtcacccatcagggcctgagctcgcccgtcacaaagagcttcaacaggggagagtgt

SEQ ID NO: 9 - protein, 452 aa, synthetic construct
  REGION 1..452: note = Description of Artificial Sequence: Syntheticpolypeptide
EVQLVESGGGLVQPGGSLRLSCAASGFTFSDYGMHWVRQAPGKGLEWVAYISSGSYTIYSADSVKGRFTISRDNAKNSLYLQMNSLRAEDTAVYYCARRAPNSFYEYYFDYWGQGTTVTVSSASTKGPSVFPLAPSSKSTSGGTAALGCLVKDYFPEPVTVSWNSGALTSGVHTFPAVLQSSGLYSLSSVVTVPSSSLGTQTYICNVNHKPSNTKVDKRVEPKSCDKTHTCPPCPAPEFEGGPSVFLFPPKPKDTLMISRTPEVTCVVVDVSHEDPEVKFNWYVDGVEVHNAKTKPREEQYNSTYRVVSVLTVLHQDWLNGKEYKCKVSNKALPASIEKTISKAKGQPREPQVCTLPPSREEMTKNQVSLSCAVKGFYPSDIAVEWESNGQPENNYKTTPPVLDSDGSFFLVSKLTVDKSRWQQGNVFSCSVMHEALHNHYTQKSLSLSPGK

SEQ ID NO: 10 - DNA, 1356 bp, synthetic construct
  misc_feature 1..1356: note = Description of Artificial Sequence: Synthetic polynucleotide
  source 1..1356: mol_type = other DNA
gaggtgcagctggtggaatccggcggaggactggtgcagcctggcggctccctgagactgtcttgcgccgcctccggcttcacattctccgactacggcatgcactgggtccgacaggcccctggaaagggcctggaatgggtggcctacatctcctccggctcctacaccatctactccgccgactccgtgaagggccggttcaccatctcccgggacaacgccaagaactccctgtacctgcagatgaactccctgcgggccgaggacacagccgtgtactactgtgccagacgggcccctaactccttctacgagtactacttcgactactggggccagggcaccaccgtgaccgtgtcctctgctagcaccaaaggtccgagcgtttttccgctggcaccgagcagcaaaagcacctctggtggcaccgcagcactgggttgtctggtgaaagattattttccggaaccggttaccgtttcttggaatagcggtgcactgaccagcggtgttcatacctttccggcagttctgcagagcagcggtctgtatagcctgtctagcgttgttaccgttccgagcagcagcctgggcacccagacctatatttgcaatgtgaatcataaaccgagcaatacaaaagttgataaacgcgttgaaccgaaaagctgtgacaaaactcacacgtgcccaccgtgcccagcacctgagttcgaggggggaccgtcagtcttcctcttccccccaaaacccaaggacaccctcatgatctcccggacccctgaggtcacatgcgtggtggtggacgtgagccacgaagaccctgaggtcaagttcaactggtacgtggacggcgtggaggtgcataatgccaagacaaagccgcgggaggagcagtacaacagcacgtaccgtgtggtcagcgtcctcaccgtcctgcaccaggactggctgaatggcaaggagtacaagtgcaaggtctccaacaaagccctcccagccagcatcgagaaaaccatctccaaagccaaagggcagccccgagaaccacaggtctgcaccctgcccccatcccgggaggagatgaccaagaaccaggtcagcctgagctgcgcggtcaaaggcttctatcccagcgacatcgccgtggagtgggagagcaatgggcagccggagaacaactacaagaccacgcctcccgtgctggactccgacggctccttcttcctcgttagcaagctcaccgtggacaagagcaggtggcagcaggggaacgtcttctcatgctccgtgatgcatgaggctctgcacaaccactacacgcagaagagcctctccctgtctccgggtaaa

SEQ ID NO: 11 - DNA, 639 bp, synthetic construct
  misc_feature 1..639: note = Description of Artificial Sequence: Synthetic polynucleotide
  source 1..639: mol_type = other DNA
gacatccagatgacccagtctccatcctccctgtctgcatctgtaggagacagagtcaccatcacttgccgggcaagtcagagcattaacagctatttagattggtatcagcagaaaccagggaaagcccctaaactcctgatctatgctgcatccagtttgcaaagtggggtcccatcaaggttcagtggcagtggatctgggacagatttcactctcaccatcagcagtctgcaacctgaagattttgcaacttactactgtcaacagtattacagtactccattcactttcggccctgggaccaaagtggaaatcaaaggtcagcccaaggcggccccctcggtcactctgttcccgccctgctctgaggagcttcaagccaacaaggccacactggtgtgtctcataagtgacttctacccgggagccgtgacagtggcctggaaggcagatagcagccccgtcaaggcgggagtggagaccaccacaccctccaaacaaagcaacaacaagtacgcggccagcagctacctgagcctgacgcctgagcagtggaagtcccacagaagctacagctgccaggtcacgcatgaagggagcaccgtggagaagacagtggcccctacagaagtgtca

SEQ ID NO: 12 - protein, 455 aa, synthetic construct
  REGION 1..455: note = Description of Artificial Sequence: Syntheticpolypeptide
QVQLVESGGGVVQPGRSLRLSCAASGFTFSSYGMHWVRQAPGKGLEWVAVIWYDGSNKYYADSVKGRFTISRDNSKNTLYLQMNSLRAEDTAVYYCARDPRGATLYYYYYGMDVWGQGTTVTVSSASTKGPSVCPLAPSSKSTSGGTAALGCLVKDYFPEPVTVSWNSGALTSGVHTFPAVLQSSGLYSLSSVVTVPSSSLGTQTYICNVNHKPSNTKVDKRVEPKSVDKTHTCPPCPAPEFEGGPSVFLFPPKPKDTLMISRTPEVTCVVVDVSHEDPEVKFNWYVDGVEVHNAKTKPREEQYNSTYRVVSVLTVLHQDWLNGKEYKCKVSNKALPASIEKTISKAKGQPREPQVYTLPPCREEMTKNQVSLWCLVKGFYPSDIAVEWESNGQPENNYKTTPPVLDSDGSFFLYSKLTVDKSRWQQGNVFSCSVMHEALHNHYTQKSLSLSPGK

SEQ ID NO: 13 - DNA, 1365 bp, synthetic construct
  misc_feature 1..1365: note = Description of Artificial Sequence: Synthetic polynucleotide
  source 1..1365: mol_type = other DNA
caggtgcagctggtggagtctgggggaggcgtggtccagcctgggaggtccctgagactctcctgtgcagcgtctggattcaccttcagtagctatggcatgcactgggtccgccaggctccaggcaaggggctggagtgggtggcagttatatggtatgatggaagtaataaatactatgcagactccgtgaagggccgattcaccatctccagagacaattccaagaacacgctgtatctgcaaatgaacagcctgagagccgaggacacggctgtgtattactgtgcgagagatccgaggggagctaccctttactactactactacggtatggacgtctggggccaagggaccacggtcaccgtctcctcagcgtcgaccaaaggtccgagcgtgtgcccgctggcaccgagcagcaaaagcacctctggtggcaccgcagcactgggttgtctggtgaaagattattttccggaaccggttaccgtttcttggaatagcggtgcactgaccagcggtgttcatacctttccggcagtcctgcagagcagcggtctgtatagcctgtctagcgttgttaccgttccgagcagcagcctgggcacccagacctatatttgcaatgtgaatcataaaccgagcaataccaaagttgataaacgcgttgaaccgaaaagcgtggacaaaactcacacgtgcccaccgtgcccagcacctgagttcgaggggggaccgtcagtcttcctcttccccccaaaacccaaggacaccctcatgatctcccggacccctgaggtcacatgcgtggtggtggacgtgagccacgaagaccctgaggtcaagttcaactggtacgtggacggcgtggaggtgcataatgccaagacaaagccgcgggaggagcagtacaacagcacgtaccgtgtggtcagcgtcctcaccgtcctgcaccaggactggctgaatggcaaggagtacaagtgcaaggtctccaacaaagccctcccagccagcatcgagaaaaccatctccaaagccaaagggcagccccgagaaccacaggtctacaccctgcccccatgccgggaggagatgaccaagaaccaggtcagcctgtggtgcctggtcaaaggcttctatcccagcgacatcgccgtggagtgggagagcaatgggcagccggagaacaactacaagaccacgcctcccgtgctggactccgacggctccttcttcctctatagcaagctcaccgtggacaagagcaggtggcagcaggggaacgtcttctcatgctccgtgatgcatgaggctctgcacaaccactacacgcagaagagcttaagcctgtctccgggtaaa

SEQ ID NO: 14 - protein, 710 aa, synthetic construct
  REGION 1..710: note = Description of Artificial Sequence: Syntheticpolypeptide
DIQMTQSPSSLSASVGDRVTITCRASQSINSYLDWYQQKPGKAPKLLIYAASSLQSGVPSRFSGSGSGTDFTLTISSLQPEDFATYYCQQYYSTPFTFGCGTKVEIKGGGGSGGGGSGGGGSGGGGSQVQLVESGGGVVQPGRSLRLSCAASGFTFSSYGMHWVRQAPGKCLEWVAVIWYDGSNKYYADSVKGRFTISRDNSKNTLYLQMNSLRAEDTAVYYCARDPRGATLYYYYYGMDVWGQGTTVTVSSGGGGSGGGGSEVQLVESGGGLVQPGGSLRLSCAASGFTFSRYWMSWVRQAPGKGLEWVANIKQDGSEKYYVDSVKGRFTISRDNAKNSLYLQMNSLRAEDTAVYYCAREGGWFGELAFDYWGQGTLVTVSSASTKGPSVFPLAPCSRSTSESTAALGCLVKDYFPEPVTVSWNSGALTSGVHTFPAVLQSSGLYSLSSVVTVPSSSLGTKTYTCNVDHKPSNTKVDKRVESKYGPPCPPCPAPEFLGGPSVFLFPPKPKDTLMISRTPEVTCVVVDVSQEDPEVQFNWYVDGVEVHNAKTKPREEQFNSTYRVVSVLTVLHQDWLNGKEYKCKVSNKGLPSSIEKTISKAKGQPREPQVYTLPPSQEEMTKNQVSLTCLVKGFYPSDIAVEWESNGQPENNYKTTPPVLDSDGSFFLYSRLTVDKSRWQEGNVFSCSVMHEALHNHYTQKSLSLSLGK

SEQ ID NO: 15 - protein, 215 aa, synthetic construct
  REGION 1..215: note = Description of Artificial Sequence: Syntheticpolypeptide
EIVLTQSPGTLSLSPGERATLSCRASQRVSSSYLAWYQQKPGQAPRLLIYDASSRATGIPDRFSGSGSGTDFTLTISRLEPEDFAVYYCQQYGSLPWTFGQGTKVEIKRTVAAPSVFIFPPSDEQLKSGTASVVCLLNNFYPREAKVQWKVDNALQSGNSQESVTEQDSKDSTYSLSSTLTLSKADYEKHKVYACEVTHQGLSSPVTKSFNRGEC

SEQ ID NO: 16 - protein, 710 aa, synthetic construct
  REGION 1..710: note = Description of Artificial Sequence: Syntheticpolypeptide
EVQLVESGGGLVQPGGSLRLSCAASGFTFSRYWMSWVRQAPGKGLEWVANIKQDGSEKYYVDSVKGRFTISRDNAKNSLYLQMNSLRAEDTAVYYCAREGGWFGELAFDYWGQGTLVTVSSASTKGPSVFPLAPCSRSTSESTAALGCLVKDYFPEPVTVSWNSGALTSGVHTFPAVLQSSGLYSLSSVVTVPSSSLGTKTYTCNVDHKPSNTKVDKRVESKYGPPCPPCPAPEFLGGPSVFLFPPKPKDTLMISRTPEVTCVVVDVSQEDPEVQFNWYVDGVEVHNAKTKPREEQFNSTYRVVSVLTVLHQDWLNGKEYKCKVSNKGLPSSIEKTISKAKGQPREPQVYTLPPSQEEMTKNQVSLTCLVKGFYPSDIAVEWESNGQPENNYKTTPPVLDSDGSFFLYSRLTVDKSRWQEGNVFSCSVMHEALHNHYTQKSLSLSLGKGGGGSGGGGSDIQMTQSPSSLSASVGDRVTITCRASQSINSYLDWYQQKPGKAPKLLIYAASSLQSGVPSRFSGSGSGTDFTLTISSLQPEDFATYYCQQYYSTPFTFGCGTKVEIKGGGGSGGGGSGGGGSGGGGSQVQLVESGGGVVQPGRSLRLSCAASGFTFSSYGMHWVRQAPGKCLEWVAVIWYDGSNKYYADSVKGRFTISRDNSKNTLYLQMNSLRAEDTAVYYCARDPRGATLYYYYYGMDVWGQGTTVTVSS

SEQ ID NO: 17 - protein, 215 aa, synthetic construct; identical to SEQ ID NO: 15
  REGION 1..215: note = Description of Artificial Sequence: Syntheticpolypeptide

SEQ ID NO: 18 - protein, 720 aa, synthetic construct
  REGION 1..720: note = Description of Artificial Sequence: Syntheticpolypeptide
EVQLVESGGGLVQPGGSLRLSCAASGFTFSRYWMSWVRQAPGKGLEWVANIKQDGSEKYYVDSVKGRFTISRDNAKNSLYLQMNSLRAEDTAVYYCAREGGWFGELAFDYWGQGTLVTVSSASTKGPSVFPLAPCSRSTSESTAALGCLVKDYFPEPVTVSWNSGALTSGVHTFPAVLQSSGLYSLSSVVTVPSSSLGTKTYTCNVDHKPSNTKVDKRVESKYGPPCPPCPAPEFLGGPSVFLFPPKPKDTLMISRTPEVTCVVVDVSQEDPEVQFNWYVDGVEVHNAKTKPREEQFNSTYRVVSVLTVLHQDWLNGKEYKCKVSNKGLPSSIEKTISKAKGQPREPQVYTLPPSQEEMTKNQVSLTCLVKGFYPSDIAVEWESNGGGGSGGGGSDIQMTQSPSSLSASVGDRVTITCRASQSINSYLDWYQQKPGKAPKLLIYAASSLQSGVPSRFSGSGSGTDFTLTISSLQPEDFATYYCQQYYSTPFTFGCGTKVEIKGGGGSGGGGSGGGGSGGGGSQVQLVESGGGVVQPGRSLRLSCAASGFTFSSYGMHWVRQAPGKCLEWVAVIWYDGSNKYYADSVKGRFTISRDNSKNTLYLQMNSLRAEDTAVYYCARDPRGATLYYYYYGMDVWGQGTTVTVSSGGGGSGGGGSGQPENNYKTTPPVLDSDGSFFLYSRLTVDKSRWQEGNVFSCSVMHEALHNHYTQKSLSLSLGK

SEQ ID NO: 19 - protein, 215 aa, synthetic construct; identical to SEQ ID NO: 15
  REGION 1..215: note = Description of Artificial Sequence: Syntheticpolypeptide

SEQ ID NO: 20 - protein, 250 aa, synthetic construct
  REGION 1..250: note = Description of Artificial Sequence: Syntheticpolypeptide
EVQLLESGGGLVQPGGSLRLSCAASGFTFSSYAMSWVRQAPGKCLEWVSAISGSGGSTYYADSVKGRFTISRDNSKNTLYLQMNSLRAEDTAVYYCARGSYGTYYGNYFEYWGRGTLVTVSSGGGGSGGGGSGGGGSGGGGSQTVLTQPPSVSVAPGKTASISCGGDNIGGKSVHWYQQKPGQAPVLVIYYDSDRPSGIPQRFSGSNSGNTATLTIHRVEAGDEADYYCQVLDRRSDHWLFGCGTKLTVL

SEQ ID NO: 21 - protein, 709 aa, synthetic construct
  REGION 1..709: note = Description of Artificial Sequence: Syntheticpolypeptide
EVQLVESGGGLVQPGGSLRLSCAASGFTFSDYGMHWVRQAPGKGLEWVAYISSGSYTIYSADSVKGRFTISRDNAKNSLYLQMNSLRAEDTAVYYCARRAPNSFYEYYFDYWGQGTTVTVSSASTKGPSVFPLAPCSRSTSESTAALGCLVKDYFPEPVTVSWNSGALTSGVHTFPAVLQSSGLYSLSSVVTVPSSSLGTKTYTCNVDHKPSNTKVDKRVESKYGPPCPPCPAPEFLGGPSVFLFPPKPKDTLMISRTPEVTCVVVDVSQEDPEVQFNWYVDGVEVHNAKTKPREEQFNSTYRVVSVLTVLHQDWLNGKEYKCKVSNKGLPSSIEKTISKAKGQPREPQVYTLPPSQEEMTKNQVSLTCLVKGFYPSDIAVEWESNGQPENNYKTTPPVLDSDGSFFLYSRLTVDKSRWQEGNVFSCSVMHEALHNHYTQKSLSLSLGKGGGGSGGGGSEVQLLESGGGLVQPGGSLRLSCAASGFTFSSYAMSWVRQAPGKCLEWVSAISGSGGSTYYADSVKGRFTISRDNSKNTLYLQMNSLRAEDTAVYYCARGSYGTYYGNYFEYWGRGTLVTVSSGGGGSGGGGSGGGGSGGGGSQTVLTQPPSVSVAPGKTASISCGGDNIGGKSVHWYQQKPGQAPVLVIYYDSDRPSGIPQRFSGSNSGNTATLTIHRVEAGDEADYYCQVLDRRSDHWLFGCGTKLTVL

SEQ ID NO: 22 - protein, 719 aa, synthetic construct
  REGION 1..719: note = Description of Artificial Sequence: Syntheticpolypeptide
EVQLVESGGGLVQPGGSLRLSCAASGFTFSDYGMHWVRQAPGKGLEWVAYISSGSYTIYSADSVKGRFTISRDNAKNSLYLQMNSLRAEDTAVYYCARRAPNSFYEYYFDYWGQGTTVTVSSASTKGPSVFPLAPCSRSTSESTAALGCLVKDYFPEPVTVSWNSGALTSGVHTFPAVLQSSGLYSLSSVVTVPSSSLGTKTYTCNVDHKPSNTKVDKRVESKYGPPCPPCPAPEFLGGPSVFLFPPKPKDTLMISRTPEVTCVVVDVSQEDPEVQFNWYVDGVEVHNAKTKPREEQFNSTYRVVSVLTVLHQDWLNGKEYKCKVSNKGLPSSIEKTISKAKGQPREPQVYTLPPSQEEMTKNQVSLTCLVKGFYPSDIAVEWESNGGGGSGGGGSEVQLLESGGGLVQPGGSLRLSCAASGFTFSSYAMSWVRQAPGKCLEWVSAISGSGGSTYYADSVKGRFTISRDNSKNTLYLQMNSLRAEDTAVYYCARGSYGTYYGNYFEYWGRGTLVTVSSGGGGSGGGGSGGGGSGGGGSQTVLTQPPSVSVAPGKTASISCGGDNIGGKSVHWYQQKPGQAPVLVIYYDSDRPSGIPQRFSGSNSGNTATLTIHRVEAGDEADYYCQVLDRRSDHWLFGCGTKLTVLGGGGSGGGGSGQPENNYKTTPPVLDSDGSFFLYSRLTVDKSRWQEGNVFSCSVMHEALHNHYTQKSLSLSLGK

SEQ ID NO: 23 - protein, 219 aa, synthetic construct; identical to SEQ ID NO: 2
  REGION 1..219: note = Description of Artificial Sequence: Syntheticpolypeptide

SEQ ID NO: 24 - protein, 709 aa, synthetic construct; identical to SEQ ID NO: 21
  REGION 1..709: note = Description of Artificial Sequence: Syntheticpolypeptide

SEQ ID NO: 25 - protein, 452 aa, synthetic construct
  REGION 1..452: note = Description of Artificial Sequence: Syntheticpolypeptide
EVQLVESGGGLVQPGGSLRLSCAASGFTFSDYGMHWVRQAPGKGLEWVAYISSGSYTIYSADSVKGRFTISRDNAKNSLYLQMNSLRAEDTAVYYCARRAPNSFYEYYFDYWGQGTTVTVSSASTKGPSVFPLAPSSKSTSGGTAALGCLVKDYFPEPVTVSWNSGALTSGVHTFPAVLQSSGLYSLSSVVTVPSSSLGTQTYICNVNHKPSNTKVDKRVEPKSCDKTHTCPPCPAPELLGGPSVFLFPPKPKDTLMISRTPEVTCVVVDVSHEDPEVKFNWYVDGVEVHNAKTKPREEQYNSTYRVVSVLTVLHQDWLNGKEYKCKVSNKALPAPIEKTISKAKGQPREPQVCTLPPSREEMTKNQVSLSCAVKGFYPSDIAVEWESNGQPENNYKTTPPVLDSDGSFFLVSKLTVDKSRWQQGNVFSCSVMHEALHNHYTQKSLSLSPGK

SEQ ID NO: 26 - protein, 214 aa, synthetic construct
  REGION 1..214: note = Description of Artificial Sequence: Syntheticpolypeptide
QTVLTQPPSVSVAPGKTASISCGGDNIGGKSVHWYQQKPGQAPVLVIYYDSDRPSGIPQRFSGSNSGNTATLTIHRVEAGDEADYYCQVLDRRSDHWLFGGGTKLTVLGQPKAAPSVTLFPPCSEELQANKATLVCLISDFYPGAVTVAWKADSSPVKAGVETTTPSKQSNNKYAASSYLSLTPEQWKSHRSYSCQVTHEGSTVEKTVAPTEVS

SEQ ID NO: 27 - protein, 451 aa, synthetic construct
  REGION 1..451: note = Description of Artificial Sequence: Syntheticpolypeptide
EVQLLESGGGLVQPGGSLRLSCAASGFTFSSYAMSWVRQAPGKGLEWVSAISGSGGSTYYADSVKGRFTISRDNSKNTLYLQMNSLRAEDTAVYYCARGSYGTYYGNYFEYWGRGTLVTVSSASTKGPSVCPLAPSSKSTSGGTAALGCLVKDYFPEPVTVSWNSGALTSGVHTFPAVLQSSGLYSLSSVVTVPSSSLGTQTYICNVNHKPSNTKVDKRVEPKSVDKTHTCPPCPAPELLGGPSVFLFPPKPKDTLMISRTPEVTCVVVDVSHEDPEVKFNWYVDGVEVHNAKTKPREEQYNSTYRVVSVLTVLHQDWLNGKEYKCKVSNKALPAPIEKTISKAKGQPREPQVYTLPPCREEMTKNQVSLWCLVKGFYPSDIAVEWESNGQPENNYKTTPPVLDSDGSFFLYSKLTVDKSRWQQGNVFSCSVMHEALHNHYTQKSLSLSPG

SEQ ID NO: 28 - protein, 214 aa, synthetic construct
  REGION 1..214: note = Description of Artificial Sequence: Syntheticpolypeptide
SYVLTQPPSVSVAPGKTARITCGGDNIGGKSVHWYQQKPGQAPVLVIYYDSDRPSGIPERFSGSNSGNTATLTISRVEAGDEADYYCQVLDRRSDHFLFGGGTKLTVLGQPKAAPSVTLFPPCSEELQANKATLVCLISDFYPGAVTVAWKADSSPVKAGVETTTPSKQSNNKYAASSYLSLTPEQWKSHRSYSCQVTHEGSTVEKTVAPTEVS

SEQ ID NO: 29 - DNA, 642 bp, synthetic construct
  misc_feature 1..642: note = Description of Artificial Sequence: Synthetic polynucleotide
  source 1..642: mol_type = other DNA
agctacgtgctgacgcagccgccgtcagtgtcagtggccccaggaaagacggccaggattacctgtgggggagacaacattggaggtaaaagtgttcactggtaccagcagaagccaggccaggcccctgtgttggtcatctattatgatagtgaccggccctcaggcatccctgagcgattctctggctccaactctgggaacacggccaccctgaccatcagcagggtcgaagccggggatgaggccgattattactgtcaggtgttggatcgtcgtagtgatcatttcctgttcggcggagggaccaagctgaccgtcctaggtcagcccaaggcggcgccctcggtcactctgttcccgccctgctctgaggagcttcaagccaacaaggccacactggtgtgtctcataagtgacttctacccgggagccgtgacagtggcctggaaggcagatagcagccccgtcaaggcgggagtggagaccaccacaccctccaaacaaagcaacaacaagtacgcggccagcagctacctgagcctgacgcctgagcagtggaagtcccacagaagctacagctgccaggtcacgcatgaagggagcaccgtggagaagacagtggcccctacagaagtgtca

SEQ ID NO: 30 - protein, 452 aa, synthetic construct
  REGION 1..452: note = Description of Artificial Sequence: Syntheticpolypeptide
EVQLLESGGGLVQPGGSLRLSCAASGFTFSSYAMSWVRQAPGKGLEWVSAISGSGGSTYYADSVKGRFTISRDNSKNTLYLQMNSLRAEDTAVYYCARGSYGTYYGNYFEYWGQGTLVTVSSASTKGPSVCPLAPSSKSTSGGTAALGCLVKDYFPEPVTVSWNSGALTSGVHTFPAVLQSSGLYSLSSVVTVPSSSLGTQTYICNVNHKPSNTKVDKRVEPKSVDKTHTCPPCPAPEFEGGPSVFLFPPKPKDTLMISRTPEVTCVVVDVSHEDPEVKFNWYVDGVEVHNAKTKPREEQYNSTYRVVSVLTVLHQDWLNGKEYKCKVSNKALPASIEKTISKAKGQPREPQVYTLPPCREEMTKNQVSLWCLVKGFYPSDIAVEWESNGQPENNYKTTPPVLDSDGSFFLYSKLTVDKSRWQQGNVFSCSVMHEALHNHYTQKSLSLSPGK

SEQ ID NO: 31 - DNA, 1356 bp, synthetic construct
  misc_feature 1..1356: note = Description of Artificial Sequence: Synthetic polynucleotide
  source 1..1356: mol_type = other DNA
gaggtgcagctgttggagtctgggggaggcttggtacagcctggggggtccctgagactctcctgtgcagcctctggattcacctttagcagctatgccatgagctgggtccgccaggctccagggaaggggctggagtgggtctcagctattagtggtagtggtggtagcacatactacgcagactccgtgaagggccggttcaccatctccagagacaattccaagaacacgctgtatctgcaaatgaacagcctgagagccgaggacacggccgtgtattactgtgcgagagggtcctatggtacctactacggaaactactttgaatactggggccagggcaccctggtcaccgtctcgagtgcgtcgaccaaaggtccgagcgtgtgcccgctggcaccgagcagcaaaagcacctctggtggcaccgcagcactgggttgtctggtgaaagattattttccggaaccggttaccgtttcttggaatagcggtgcactgaccagcggtgttcatacctttccggcagtcctgcagagcagcggtctgtatagcctgtctagcgttgttaccgttccgagcagcagcctgggcacccagacctatatttgcaatgtgaatcataaaccgagcaataccaaagttgataaacgcgttgaaccgaaaagcgtggacaaaactcacacgtgcccaccgtgcccagcacctgagttcgaggggggaccgtcagtcttcctcttccccccaaaacccaaggacaccctcatgatctcccggacccctgaggtcacatgcgtggtggtggacgtgagccacgaagaccctgaggtcaagttcaactggtacgtggacggcgtggaggtgcataatgccaagacaaagccgcgggaggagcagtacaacagcacgtaccgtgtggtcagcgtcctcaccgtcctgcaccaggactggctgaatggcaaggagtacaagtgcaaggtctccaacaaagccctcccagccagcatcgagaaaaccatctccaaagccaaagggcagccccgagaaccacaggtctacaccctgcccccatgccgggaggagatgaccaagaaccaggtcagcctgtggtgcctggtcaaaggcttctatcccagcgacatcgccgtggagtgggagagcaatgggcagccggagaacaactacaagaccacgcctcccgtgctggactccgacggctccttcttcctctatagcaagctcaccgtggacaagagcaggtggcagcaggggaacgtcttctcatgctccgtgatgcatgaggctctgcacaaccactacacgcagaagagcttaagcctgtctccgggtaaa

SEQ ID NO: 32 - protein, 214 aa, synthetic construct
  REGION 1..214: note = Description of Artificial Sequence: Syntheticpolypeptide
DIQMTQSPSSLSASVGDRVTITCRASQDISNYLNWYQQKPGKAPKLLIYYTSKLHSGVPSRFSGSGSGTDYTLTISSLQPEDFATYYCQQGSALPWTFGQGTKVEIKRTVAAPSVFIFPPSDEQLKSGTASVVCLLNNFYPREAKVQWKVDNALQSGNSQESVTEQDSKDSTYSLSSTLTLSKADYEKHKVYACEVTHQGLSSPVTKSFNRGEC

SEQ ID NO: 33 - protein, 215 aa, synthetic construct; identical to SEQ ID NO: 15
  REGION 1..215: note = Description of Artificial Sequence: Syntheticpolypeptide

SEQ ID NO: 34 - protein, 707 aa, synthetic construct
  REGION 1..707: note = Description of Artificial Sequence: Syntheticpolypeptide
EIVLTQSPGTLSLSPGERATLSCRASQRVSSSYLAWYQQKPGQAPRLLIYDASSRATGIPDRFSGSGSGTDFTLTISRLEPEDFAVYYCQQYGSLPWTFGCGTKVEIKGGGGSGGGGSGGGGSGGGGSEVQLVESGGGLVQPGGSLRLSCAASGFTFSRYWMSWVRQAPGKCLEWVANIKQDGSEKYYVDSVKGRFTISRDNAKNSLYLQMNSLRAEDTAVYYCAREGGWFGELAFDYWGQGTLVTVSSGGGGSGGGGSQVQLQESGPGLVKPSQTLSLTCAVYGGSFSSGYWNWIRKHPGKGLEYIGYISYNGITYHNPSLKSRITINRDTSKNQYSLQLNSVTPEDTAVYYCARYKYDYDGGHAMDYWGQGTLVTVSSASTKGPSVFPLAPCSRSTSESTAALGCLVKDYFPEPVTVSWNSGALTSGVHTFPAVLQSSGLYSLSSVVTVPSSSLGTKTYTCNVDHKPSNTKVDKRVESKYGPPCPPCPAPEFLGGPSVFLFPPKPKDTLMISRTPEVTCVVVDVSQEDPEVQFNWYVDGVEVHNAKTKPREEQFNSTYRVVSVLTVLHQDWLNGKEYKCKVSNKGLPSSIEKTISKAKGQPREPQVYTLPPSQEEMTKNQVSLTCLVKGFYPSDIAVEWESNGQPENNYKTTPPVLDSDGSFFLYSRLTVDKSRWQEGNVFSCSVMHEALHNHYTQKSLSLSLGK

SEQ ID NO: 35 - protein, 707 aa, synthetic construct
  REGION 1..707: note = Description of Artificial Sequence: Syntheticpolypeptide
QVQLQESGPGLVKPSQTLSLTCAVYGGSFSSGYWNWIRKHPGKGLEYIGYISYNGITYHNPSLKSRITINRDTSKNQYSLQLNSVTPEDTAVYYCARYKYDYDGGHAMDYWGQGTLVTVSSASTKGPSVFPLAPCSRSTSESTAALGCLVKDYFPEPVTVSWNSGALTSGVHTFPAVLQSSGLYSLSSVVTVPSSSLGTKTYTCNVDHKPSNTKVDKRVESKYGPPCPPCPAPEFLGGPSVFLFPPKPKDTLMISRTPEVTCVVVDVSQEDPEVQFNWYVDGVEVHNAKTKPREEQFNSTYRVVSVLTVLHQDWLNGKEYKCKVSNKGLPSSIEKTISKAKGQPREPQVYTLPPSQEEMTKNQVSLTCLVKGFYPSDIAVEWESNGQPENNYKTTPPVLDSDGSFFLYSRLTVDKSRWQEGNVFSCSVMHEALHNHYTQKSLSLSLGKGGGGSGGGGSEIVLTQSPGTLSLSPGERATLSCRASQRVSSSYLAWYQQKPGQAPRLLIYDASSRATGIPDRFSGSGSGTDFTLTISRLEPEDFAVYYCQQYGSLPWTFGCGTKVEIKGGGGSGGGGSGGGGSGGGGSEVQLVESGGGLVQPGGSLRLSCAASGFTFSRYWMSWVRQAPGKCLEWVANIKQDGSEKYYVDSVKGRFTISRDNAKNSLYLQMNSLRAEDTAVYYCAREGGWFGELAFDYWGQGTLVTVSS

SEQ ID NO: 36 - protein, 707 aa, synthetic construct; identical to SEQ ID NO: 35
  REGION 1..707: note = Description of Artificial Sequence: Syntheticpolypeptide

SEQ ID NO: 37 - protein, 718 aa, synthetic construct
  REGION 1..718: note = Description of Artificial Sequence: Syntheticpolypeptide
EVQLVESGGGLVQPGGSLRLSCAASGFTFSSHDMHWVRQATGKGLEWVSGIGTAGDTYYPDSVKGRFTISRENAKNSLYLQMNSLRAGDTAVYYCARDRYSPTGHYYGMDVWGQGTTVTVSSASTKGPSVFPLAPSSKSTSGGTAALGCLVKDYFPEPVTVSWNSGALTSGVHTFPAVLQSSGLYSLSSVVTVPSSSLGTQTYICNVNHKPSNTKVDKRVEPKSCDKTHTCPPCPAPELLGGPSVFLFPPKPKDTLMISRTPEVTCVVVDVSHEDPEVKFNWYVDGVEVHNAKTKPREEQYNSTYRVVSVLTVLHQDWLNGKEYKCKVSNKALPAPIEKTISKAKGQPREPQVYTLPPSREEMTKNQVSLTCLVKGFYPSDIAVEWESNGGGGSGGGGSEIVMTQSPATLSVSPGERATLSCRASQSVSSYLGWYQQKPGQAPRLLIYGASTRATGIPARFSGSGSGTEFTLTISSLQSEDFAVYYCQQYQNWPLLTFGCGTKLEIKGGGGSGGGGSGGGGSGGGGSEVQLLESGGGLVQPGGSLRLSCAASGFTFSPYMMQWVRQAPGKCLEWVSSIWPSGGKTYYADSVKGRFTISRDNSKNTLYLQMNSLRAEDTAVYYCARVRRGGATDYWGQGTLVTVSSGGGGSGGGGSGQPENNYKTTPPVLDSDGSFFLYSKLTVDKSRWQQGNVFSCSVMHEALHNHYTQKSLSLSPGK

SEQ ID NO: 38 - protein, 716 aa, synthetic construct
  REGION 1..716: note = Description of Artificial Sequence: Syntheticpolypeptide
EVQLLESGGGLVQPGGSLRLSCAASGFTFSPYMMQWVRQAPGKGLEWVSSIWPSGGKTYYADSVKGRFTISRDNSKNTLYLQMNSLRAEDTAVYYCARVRRGGATDYWGQGTLVTVSSASTKGPSVFPLAPSSKSTSGGTAALGCLVKDYFPEPVTVSWNSGALTSGVHTFPAVLQSSGLYSLSSVVTVPSSSLGTQTYICNVNHKPSNTKVDKRVEPKSCDKTHTCPPCPAPELLGGPSVFLFPPKPKDTLMISRTPEVTCVVVDVSHEDPEVKFNWYVDGVEVHNAKTKPREEQYNSTYRVVSVLTVLHQDWLNGKEYKCKVSNKALPAPIEKTISKAKGQPREPQVYTLPPSREEMTKNQVSLTCLVKGFYPSDIAVEWESNGGGGSGGGGSDIQMTQSPSTLSASVGDRVTITCRASQSISSWLAWYQQKPGKAPKLLIYKASSLESGVPSRFSGSGSGTEFTLTISSLQPDDFATYYCKQYADYWTFGCGTKVEIKGGGGSGGGGSGGGGSGGGGSEVQLVESGGGLVQPGGSLRLSCAASGFTFSSHDMHWVRQATGKCLEWVSGIGTAGDTYYPDSVKGRFTISRENAKNSLYLQMNSLRAGDTAVYYCARDRYSPTGHYYGMDVWGQGTTVTVSSGGGGSGGGGSGQPENNYKTTPPVLDSDGSFFLYSKLTVDKSRWQQGNVFSCSVMHEALHNHYTQKSLSLSPGK

SEQ ID NO: 39 - protein, 5 aa, synthetic construct
  REGION 1..5: note = Description of Artificial Sequence: Syntheticpolypeptide
ISRTP

SEQ ID NO: 40 - protein, 5 aa, synthetic construct
  REGION 1..5: note = Description of Artificial Sequence: Syntheticpolypeptide
AKGQP

SEQ ID NO: 41 - protein, 10 aa, synthetic construct
  REGION 1..10: note = Description of Artificial Sequence: Syntheticpolypeptide
GGGGSGGGGS

SEQ ID NO: 42 - protein, 15 aa, synthetic construct
  REGION 1..15: note = Description of Artificial Sequence: Syntheticpolypeptide
GGGGSGGGGSGGGGS

SEQ ID NO: 43 - protein, 20 aa, synthetic construct
  REGION 1..20: note = Description of Artificial Sequence: Syntheticpolypeptide
GGGGSGGGGSGGGGSGGGGS

SEQ ID NO: 44 - protein, 15 aa, synthetic construct
  REGION 1..15: note = Description of Artificial Sequence: Syntheticpolypeptide
EPKSCDKTHTCPPCP

SEQ ID NO: 45 - protein, 8 aa, synthetic construct
  REGION 1..8: note = Description of Artificial Sequence: Syntheticpolypeptide
EPKSCDKT

SEQ ID NO: 46 - protein, 8 aa, synthetic construct
  REGION 1..8: note = Description of Artificial Sequence: Syntheticpolypeptide
EPKSCGKT

SEQ ID NO: 47 - protein, 5 aa, synthetic construct
  REGION 1..5: note = Description of Artificial Sequence: Syntheticpolypeptide
EPKSC

SEQ ID NO: 48 - protein, 5 aa, synthetic construct
  REGION 1..5: note = Description of Artificial Sequence: Syntheticpolypeptide
GGGGS

SEQ ID NO: 49 - protein, 112 aa, synthetic construct
  REGION 1..112: note = Description of Artificial Sequence: Syntheticpolypeptide
QIVLTQSPATLSLSPGERATLSCSASSKHTNLYWSRHMYWYQQKPGQAPRLLIYLTSNRATGIPARFSGSGSGTDFTLTISSLEPEDFAVYYCQQWSSNPFTFGQGTKLEIK

SEQ ID NO: 50 - protein, 449 aa, synthetic construct
  REGION 1..449: note = Description of Artificial Sequence: Syntheticpolypeptide
EVQLVESGGGLVQPGGSLRLSCAASGFTFSDYGMHWVRQAPGKGLEWVAYISSGSYTIYSADSVKGRFTISRDNAKNSLYLQMNSLRAEDTAVYYCARRAPNSFYEYYFDYWGQGTTVTVSSASTKGPSVFPLAPCSRSTSESTAALGCLVKDYFPEPVTVSWNSGALTSGVHTFPAVLQSSGLYSLSSVVTVPSSSLGTKTYTCNVDHKPSNTKVDKRVESKYGPPCPPCPAPEFLGGPSVFLFPPKPKDTLMISRTPEVTCVVVDVSQEDPEVQFNWYVDGVEVHNAKTKPREEQFNSTYRVVSVLTVLHQDWLNGKEYKCKVSNKGLPSSIEKTISKAKGQPREPQVYTLPPSQEEMTKNQVSLTCLVKGFYPSDIAVEWESNGQPENNYKTTPPVLDSDGSFFLYSRLTVDKSRWQEGNVFSCSVMHEALHNHYTQKSLSLSLGK

SEQ ID NO: 51 - protein, 122 aa, synthetic construct
  REGION 1..122: note = Description of Artificial Sequence: Syntheticpolypeptide
EVQLVESGGGLVQPGGSLRLSCAASGFTFSDYGMHWVRQAPGKGLEWVAYISSGSYTIYSADSVKGRFTISRDNAKNSLYLQMNSLRAEDTAVYYCARRAPNSFYEYYFDYWGQGTTVTVSS

SEQ ID NO: 52 - protein, 125 aa, synthetic construct
  REGION 1..125: note = Description of Artificial Sequence: Syntheticpolypeptide
QVQLVESGGGVVQPGRSLRLSCAASGFTFSSYGMHWVRQAPGKGLEWVAVIWYDGSNKYYADSVKGRFTISRDNSKNTLYLQMNSLRAEDTAVYYCARDPRGATLYYYYYGMDVWGQGTTVTVSS

SEQ ID NO: 53 - protein, 167 aa, synthetic construct
  REGION 1..167: note = CTLA-4 HC
GVVQPGRSLRLSCAASGFTFSSYGMHWVRQAPGKGLEWVAVIWYDGSNKYYADSVKGRFTISRDNSKNTLYLQMNSLRAEDTAVYYCARDPRGATLYYYYYGMDVWGQGTTVTVSSASTKGPSVFPLAPCSRSTSESTAALGCLVKDYFPEPVTVSWNSGALTSGVH

SEQ ID NO: 54 - protein, 107 aa, synthetic construct
  REGION 1..107: note = Description of Artificial Sequence: Syntheticpolypeptide
DIQMTQSPSSLSASVGDRVTITCRASQSINSYLDWYQQKPGKAPKLLIYAASSLQSGVPSRFSGSGSGTDFTLTISSLQPEDFATYYCQQYYSTPFTFGPGTKVEIK

SEQ ID NO: 55 - protein, 214 aa, synthetic construct
  REGION 1..214: note = Description of Artificial Sequence: Syntheticpolypeptide
DIQMTQSPSSLSASVGDRVTITCRASQSINSYLDWYQQKPGKAPKLLIYAASSLQSGVPSRFSGSGSGTDFTLTISSLQPEDFATYYCQQYYSTPFTFGPGTKVEIKRTVAAPSVFIFPPSDEQLKSGTASVVCLLNNFYPREAKVQWKVDNALQSGNSQESVTEQDSKDSTYSLSSTLTLSKADYEKHKVYACEVTHQGLSSPVTKSFNRGEC

SEQ ID NO: 56 - protein, 114 aa, synthetic construct
  REGION 1..114: note = Description of Artificial Sequence: Syntheticpolypeptide
EVQLVESGGGLVQPGRSLRLSCTASGYTFPDYYMNWVRQAPGKGLEWVGDIDPNYGGTTYNASVKGRFTISVDRSKSIAYLQMSSLKTEDTAVYYCARGALTDWGQGTMVTVSS

SEQ ID NO: 57 - protein, 213 aa, synthetic construct
  REGION 1..213: note = Description of Artificial Sequence: Syntheticpolypeptide
QIQLTQSPSILSASVGDRVTITCRASSSVSYIYWFQQKPGKAPKPLIYATFNLASGVPSRFSGSGSGTSYTLTISSLQPEDFATYYCQQWSNNPLTFGQGTKVEIKRTVAAPSVFIFPPSDEQLKSGTASVVCLLNNFYPREAKVQWKVDNALQSGNSQESVTEQDSKDSTYSLSSTLTLSKADYEKHKVYACEVTHQGLSSPVTKSFNRGEC

SEQ ID NO: 58 - protein, 106 aa, synthetic construct
  REGION 1..106: note = Description of Artificial Sequence: Syntheticpolypeptide
QIQLTQSPSILSASVGDRVTITCRASSSVSYIYWFQQKPGKAPKPLIYATFNLASGVPSRFSGSGSGTSYTLTISSLQPEDFATYYCQQWSNNPLTFGQGTKVEIK

SEQ ID NO: 59 - protein, 121 aa, synthetic construct
  REGION 1..121: note = Description of Artificial Sequence: Syntheticpolypeptide
EVQLVESGGGLVQPGGSLRLSCAASGFTFSRYWMSWVRQAPGKGLEWVANIKQDGSEKYYVDSVKGRFTISRDNAKNSLYLQMNSLRAEDTAVYYCAREGGWFGELAFDYWGQGTLVTVSS

SEQ ID NO: 60 - protein, 108 aa, synthetic construct
  REGION 1..108: note = Description of Artificial Sequence: Syntheticpolypeptide
EIVLTQSPGTLSLSPGERATLSCRASQRVSSSYLAWYQQKPGQAPRLLIYDASSRATGIPDRFSGSGSGTDFTLTISRLEPEDFAVYYCQQYGSLPWTFGQGTKVEIK

SEQ ID NO: 61 - protein, 214 aa, synthetic construct
  REGION 1..214: note = Description of Artificial Sequence: Syntheticpolypeptide
QTVLTQPPSVSVAPGKTASISCGGDNIGGKSVHWYQQKPGQAPVLVIYYDSDRPSGIPQRFSGSNSGNTATLTIHRVEAGDEADYYCQVLDRRSDHWLFGGGTKLTVLGQPKAAPSVTLFPPSSEELQANKATLVCLISDFYPGAVTVAWKADSSPVKAGVETTTPSKQSNNKYAASSYLSLTPEQWKSHRSYSCQVTHEGSTVEKTVAPTECS

SEQ ID NO: 62 - protein, 108 aa, synthetic construct
  REGION 1..108: note = Description of Artificial Sequence: Syntheticpolypeptide
QTVLTQPPSVSVAPGKTASISCGGDNIGGKSVHWYQQKPGQAPVLVIYYDSDRPSGIPQRFSGSNSGNTATLTIHRVEAGDEADYYCQVLDRRSDHWLFGGGTKLTVL

SEQ ID NO: 63 - protein, 449 aa, synthetic construct
  REGION 1..449: note = Description of Artificial Sequence: Syntheticpolypeptide
EVQLLESGGGLVQPGGSLRLSCAASGFTFSSYAMSWVRQAPGKGLEWVSAISGSGGSTYYADSVKGRFTISRDNSKNTLYLQMNSLRAEDTAVYYCARGSYGTYYGNYFEYWGRGTLVTVSSASTKGPSVFPLAPCSRSTSESTAALGCLVKDYFPEPVTVSWNSGALTSGVHTFPAVLQSSGLYSLSSVVTVPSSSLGTKTYTCNVDHKPSNTKVDKRVESKYGPPCPPCPAPEFLGGPSVFLFPPKPKDTLMISRTPEVTCVVVDVSQEDPEVQFNWYVDGVEVHNAKTKPREEQFNSTYRVVSVLTVLHQDWLNGKEYKCKVSNKGLPSSIEKTISKAKGQPREPQVYTLPPSQEEMTKNQVSLTCLVKGFYPSDIAVEWESNGQPENNYKTTPPVLDSDGSFFLYSRLTVDKSRWQEGNVFSCSVMHEALHNHYTQKSLSLSLGK

SEQ ID NO: 64 - protein, 122 aa, synthetic construct
  REGION 1..122: note = Description of Artificial Sequence: Syntheticpolypeptide
EVQLLESGGGLVQPGGSLRLSCAASGFTFSSYAMSWVRQAPGKGLEWVSAISGSGGSTYYADSVKGRFTISRDNSKNTLYLQMNSLRAEDTAVYYCARGSYGTYYGNYFEYWGRGTLVTVSS

SEQ ID NO: 65 - protein, 214 aa, synthetic construct
  REGION 1..214: note = Description of Artificial Sequence: Syntheticpolypeptide
SYVLTQPPSVSVAPGKTARITCGGDNIGGKSVHWYQQKPGQAPVLVIYYDSDRPSGIPERFSGSNSGNTATLTISRVEAGDEADYYCQVLDRRSDHWLFGGGTKLTVLGQPKAAPSVTLFPPSSEELQANKATLVCLISDFYPGAVTVAWKADSSPVKAGVETTTPSKQSNNKYAASSYLSLTPEQWKSHRSYSCQVTHEGSTVEKTVAPTECS

SEQ ID NO: 66 - protein, 108 aa, synthetic construct
  REGION 1..108: note = Description of Artificial Sequence: Syntheticpolypeptide
SYVLTQPPSVSVAPGKTARITCGGDNIGGKSVHWYQQKPGQAPVLVIYYDSDRPSGIPERFSGSNSGNTATLTISRVEAGDEADYYCQVLDRRSDHWLFGGGTKLTVL

SEQ ID NO: 67 - protein, 449 aa, synthetic construct
  REGION 1..449: note = Description of Artificial Sequence: Syntheticpolypeptide
EVQLLESGGGLVQPGGSLRLSCAASGFTFSSYAMSWVRQAPGKGLEWVSAISGSGGSTYYADSVKGRFTISRDNSKNTLYLQMNSLRAEDTAVYYCARGSYGTYYGNYFEYWGQGTLVTVSSASTKGPSVFPLAPCSRSTSESTAALGCLVKDYFPEPVTVSWNSGALTSGVHTFPAVLQSSGLYSLSSVVTVPSSSLGTKTYTCNVDHKPSNTKVDKRVESKYGPPCPPCPAPEFLGGPSVFLFPPKPKDTLMISRTPEVTCVVVDVSQEDPEVQFNWYVDGVEVHNAKTKPREEQFNSTYRVVSVLTVLHQDWLNGKEYKCKVSNKGLPSSIEKTISKAKGQPREPQVYTLPPSQEEMTKNQVSLTCLVKGFYPSDIAVEWESNGQPENNYKTTPPVLDSDGSFFLYSRLTVDKSRWQEGNVFSCSVMHEALHNHYTQKSLSLSLGK

SEQ ID NO: 68 - protein, 122 aa, synthetic construct
  REGION 1..122: note = Description of Artificial Sequence: Syntheticpolypeptide
EVQLLESGGGLVQPGGSLRLSCAASGFTFSSYAMSWVRQAPGKGLEWVSAISGSGGSTYYADSVKGRFTISRDNSKNTLYLQMNSLRAEDTAVYYCARGSYGTYYGNYFEYWGQGTLVTVSS

SEQ ID NO: 69 - protein, 121 aa, synthetic construct
  REGION 1..121: note = Description of Artificial Sequence: Syntheticpolypeptide
QVQLQESGPGLVKPSQTLSLTCAVYGGSFSSGYWNWIRKHPGKGLEYIGYISYNGITYHNPSLKSRITINRDTSKNQYSLQLNSVTPEDTAVYYCARYKYDYDGGHAMDYWGQGTLVTVSS

SEQ ID NO: 70 - protein, 107 aa, synthetic construct
  REGION 1..107: note = Description of Artificial Sequence: Syntheticpolypeptide
DIQMTQSPSSLSASVGDRVTITCRASQDISNYLNWYQQKPGKAPKLLIYYTSKLHSGVPSRFSGSGSGTDYTLTISSLQPEDFATYYCQQGSALPWTFGQGTKVEIK

SEQ ID NO: 71 - protein, 451 aa, synthetic construct
  REGION 1..451: note = Description of Artificial Sequence: Syntheticpolypeptide
QVQLQESGPGLVKPSQTLSLTCAVYGGSFSSGYWNWIRKHPGKGLEYIGYISYNGITYHNPSLKSRITINRDTSKNQYSLQLNSVTPEDTAVYYCARYKYDYDGGHAMDYWGQGTLVTVSSASTKGPSVFPLAPSSKSTSGGTAALGCLVKDYFPEPVTVSWNSGALTSGVHTFPAVLQSSGLYSLSSVVTVPSSSLGTQTYICNVNHKPSNTKVDKRVEPKSCDKTHTCPPCPAPELLGGPSVFLFPPKPKDTLMISRTPEVTCVVVDVSHEDPEVKFNWYVDGVEVHNAKTKPREEQYNSTYRVVSVLTVLHQDWLNGKEYKCKVSNKALPAPIEKTISKAKGQPREPQVYTLPPSREEMTKNQVSLTCLVKGFYPSDIAVEWESNGQPENNYKTTPPVLDSDGSFFLYSKLTVDKSRWQQGNVFSCSVMHEALHNHYTQKSLSLSPGK

SEQ ID NO: 72 - protein, 214 aa, synthetic construct; identical to SEQ ID NO: 32
  REGION 1..214: note = Description of Artificial Sequence: Syntheticpolypeptide

SEQ ID NO: 73 - protein, 288 aa, Homo sapiens
MQIPQAPWPVVWAVLQLGWRPGWFLDSPDRPWNPPTFSPALLVVTEGDNATFTCSFSNTSESFVLNWYRMSPSNQTDKLAAFPEDRSQPGQDCRFRVTQLPNGRDFHMSVVRARRNDSGTYLCGAISLAPKAQIKESLRAELRVTERRAEVPTAHPSPSPRPAGQFQTLVVGVVGGLLGSLVLLVWVLAVICSRAARGTIGARRTGQPLKEDPSAVPVFSVDYGELDFQWREKTPEPPVPCVPEQTEYATIVFPSGMGTSSPARRGSADGPRSAQPLRPEDGHCSWPL

SEQ ID NO: 74 - protein, 176 aa, Homo sapiens
MRIFAVFIFMTYWHLLNAPYNKINQRILVVDPVTSEHELTCQAEGYPKAEVIWTSSDHQVLSGKTTTTNSKREEKLFNVTSTLRINTTTNEIFYCTFRRLDPEENHTAELVIPELPLAHPPNERTHLVILGAILLCLGVALTFIFRLRKGRMMDVKKCGIQDTNSKKQSDTHLEET

SEQ ID NO: 75 - protein, 223 aa, Homo sapiens
MACLGFQRHKAQLNLATRTWPCTLLFFLLFIPVFCKAMHVAQPAVVLASSRGIASFVCEYASPGKATEVRVTVLRQADSQVTEVCAATYMMGNELTFLDDSICTGTSSGNQVNLTIQGLRAMDTGLYICKVELMYPPPYYLGIGNGTQIYVIDPEPCPDSDFLLWILAAVSSGLFFYSFLLTAVSLSKMLKKRSPLTTGVYVKMPPTEPECEKQFQPYFIPIN

SEQ ID NO: 76 - protein, 301 aa, Homo sapiens
MFSHLPFDCVLLLLLLLLTRSSEVEYRAEVGQNAYLPCFYTPAAPGNLVPVCWGKGACPVFECGNVVLRTDERDVNYWTSRYWLNGDFRKGDVSLTIENVTLADSGIYCCRIQIPGIMNDEKFNLKLVIKPAKVTPAPTRQRDFTAAFPRMLTTRGHGPAETQTLGSLPDINLTQISTLANELRDSRLANDLRDSGATIRIGIYIGAGICAGLALALIFGALIFKWYSHSKEKIQNLSLISLANLPPSGLANAVAEGIRSEENIYTIEENVYEVEEPNEYYCYVSSRQQPSQPLGCRFAMP

SEQ ID NO: 77 - protein, 278 aa, Homo sapiens
MGSPGMVLGLLVQIWALQEASSLSVQQGPNLLQVRQGSQATLVCQVDQATAWERLRVKWTKDGAILCQPYITNGSLSLGVCGPQGRLSWQAPSHLTLQLDPVSLNHSGAYVCWAAVEIPELEEAEGNITRLFVDPDDPTQNRNRIASFPGFLFVLLGVGSMGVAAIVWGAWFWGRRSCQQRDSGNAFYSNVLYRPRGAPKKSEDCSGEGKDQRGQSIYSTSFPQPAPRQPHLASRPCPSPRPCPSPRPGHPVSMVRVSPRPSPTQQPRPKGFPKVGEE

SEQ ID NO: 78 - protein, 277 aa, Homo sapiens
MCVGARRLGRGPCAALLLLGLGLSTVTGLHCVGDTYPSNDRCCHECRPGNGMVSRCSRSQNTVCRPCGPGFYNDVVSSKPCKPCTWCNLRSGSERKQLCTATQDTVCRCRAGTQPLDSYKPGVDCAPCPPGHFSPGDNQACKPWTNCTLAGKHTLQPASNSSDAICEDRDPPATQPQETQGPPARPITVQPTEAWPRTSQGPSTRPVEVPGGRAVAAILGLGLVLGLLGPLAILLALYLLRRDQRLPPDAHKPPGGGSFRTPIQEEQADAHSTLAKI

SEQ ID NO: 79 - protein, 10 aa, synthetic construct
  REGION 1..10: note = Description of Artificial Sequence: Syntheticpolypeptide
GFTFSSYAMS

SEQ ID NO: 80 - protein, 17 aa, synthetic construct
  REGION 1..17: note = Description of Artificial Sequence: Syntheticpolypeptide
AISGSGGSTYYADSVKG

SEQ ID NO: 81 - protein, 13 aa, synthetic construct
  REGION 1..13: note = Description of Artificial Sequence: Syntheticpolypeptide
GSYGTYYGNYFEY

SEQ ID NO: 82 - protein, 11 aa, synthetic construct
  REGION 1..11: note = Description of Artificial Sequence: Syntheticpolypeptide
GGDNIGGKSVH

SEQ ID NO: 83 - protein, 7 aa, synthetic construct
  REGION 1..7: note = Description of Artificial Sequence: Syntheticpolypeptide
YDSDRPS

SEQ ID NO: 84 - protein, 9 aa, synthetic construct
  REGION 1..9: note = Description of Artificial Sequence: Syntheticpolypeptide
QVLDRRSDH

SEQ ID NO: 85 - protein, 122 aa, synthetic construct; identical to SEQ ID NO: 64
  REGION 1..122: note = Description of Artificial Sequence: Syntheticpolypeptide

SEQ ID NO: 86 - protein, 108 aa, synthetic construct; identical to SEQ ID NO: 62
  REGION 1..108: note = Description of Artificial Sequence: Syntheticpolypeptide

SEQ ID NO: 87 - protein, 449 aa, synthetic construct; identical to SEQ ID NO: 63
  REGION 1..449: note = Description of Artificial Sequence: Syntheticpolypeptide

SEQ ID NO: 88 - protein, 214 aa, synthetic construct; identical to SEQ ID NO: 61
  REGION 1..214: note = Description of Artificial Sequence: Syntheticpolypeptide

SEQ ID NO: 89 - protein, 712 aa, synthetic construct
  REGION 1..712: note = BiS3 PD-1(LO115)/TIM3(O13-1) HC
EVQLVESGGGLVQPGGSLRLSCAASGFTFSDYGMHWVRQAPGKGLEWVAYISSGSYTIYSADSVKGRFTISRDNAKNSLYLQMNSLRAEDTAVYYCARRAPNSFYEYYFDYWGQGTTVTVSSASTKGPSVFPLAPSSKSTSGGTAALGCLVKDYFPEPVTVSWNSGALTSGVHTFPAVLQSSGLYSLSSVVTVPSSSLGTQTYICNVNHKPSNTKVDKRVEPKSCDKTHTCPPCPAPEFEGGPSVFLFPPKPKDTLMISRTPEVTCVVVDVSHEDPEVKFNWYVDGVEVHNAKTKPREEQYNSTYRVVSVLTVLHQDWLNGKEYKCKVSNKALPASIEKTISKAKGQPREPQVYTLPPSREEMTKNQVSLTCLVKGFYPSDIAVEWESNGQPENNYKTTPPVLDSDGSFFLYSKLTVDKSRWQQGNVFSCSVMHEALHNHYTQKSLSLSPGKGGGGSGGGGSEVQLLESGGGLVQPGGSLRLSCAASGFTFSSYAMSWVRQAPGKCLEWVSAISGSGGSTYYADSVKGRFTISRDNSKNTLYLQMNSLRAEDTAVYYCARGSYGTYYGNYFEYWGQGTLVTVSSGGGGSGGGGSGGGGSGGGGSSYVLTQPPSVSVAPGKTARITCGGDNIGGKSVHWYQQKPGQAPVLVIYYDSDRPSGIPERFSGSNSGNTATLTISRVEAGDEADYYCQVLDRRSDHFLFGCGTKLTVL

SEQ ID NO: 90 - protein, 219 aa, synthetic construct; identical to SEQ ID NO: 2
  REGION 1..219: note = BiS3 PD-1(LO115)/TIM3(O13-1) LC

SEQ ID NO: 91 - protein, 722 aa, synthetic construct
  REGION 1..722: note = BiS5 PD-1(LO115)/TIM3(O13-1) HC
EVQLVESGGGLVQPGGSLRLSCAASGFTFSDYGMHWVRQAPGKGLEWVAYISSGSYTIYSADSVKGRFTISRDNAKNSLYLQMNSLRAEDTAVYYCARRAPNSFYEYYFDYWGQGTTVTVSSASTKGPSVFPLAPSSKSTSGGTAALGCLVKDYFPEPVTVSWNSGALTSGVHTFPAVLQSSGLYSLSSVVTVPSSSLGTQTYICNVNHKPSNTKVDKRVEPKSCDKTHTCPPCPAPEFEGGPSVFLFPPKPKDTLMISRTPEVTCVVVDVSHEDPEVKFNWYVDGVEVHNAKTKPREEQYNSTYRVVSVLTVLHQDWLNGKEYKCKVSNKALPASIEKTISKAKGQPREPQVYTLPPSREEMTKNQVSLTCLVKGFYPSDIAVEWESNGGGGSGGGGSEVQLLESGGGLVQPGGSLRLSCAASGFTFSSYAMSWVRQAPGKCLEWVSAISGSGGSTYYADSVKGRFTISRDNSKNTLYLQMNSLRAEDTAVYYCARGSYGTYYGNYFEYWGQGTLVTVSSGGGGSGGGGSGGGGSGGGGSSYVLTQPPSVSVAPGKTARITCGGDNIGGKSVHWYQQKPGQAPVLVIYYDSDRPSGIPERFSGSNSGNTATLTISRVEAGDEADYYCQVLDRRSDHFLFGCGTKLTVLGGGGSGGGGSGQPENNYKTTPPVLDSDGSFFLYSKLTVDKSRWQQGNVFSCSVMHEALHNHYTQKSLSLSPGK

SEQ ID NO: 92 - protein, 219 aa, synthetic construct; identical to SEQ ID NO: 2
  REGION 1..219: note = BiS5 PD-1(LO115)/TIM3(O13-1) LC

SEQ ID NO: 93 - protein, 214 aa, synthetic construct; identical to SEQ ID NO: 32
  REGION 1..214: note = OX40SLR LCv kappa

SEQ ID NO: 94 - protein, 720 aa, synthetic construct
  REGION 1..720: note = BiS5-OX40SLR HC-G1-N434A-PD-L1
QVQLQESGPGLVKPSQTLSLTCAVYGGSFSSGYWNWIRKHPGKGLEYIGYISYNAITYHNPSLKSRITINRDTSKNQYSLQLNSVTPEDTAVYYCARYKYDYEGGHAMDYWGQGTLVTVSSASTKGPSVFPLAPSSKSTSGGTAALGCLVKDYFPEPVTVSWNSGALTSGVHTFPAVLQSSGLYSLSSVVTVPSSSLGTQTYICNVNHKPSNTKVDKRVEPKSCDKTHTCPPCPAPELLGGPSVFLFPPKPKDTLMISRTPEVTCVVVDVSHEDPEVKFNWYVDGVEVHNAKTKPREEQYNSTYRVVSVLTVLHQDWLNGKEYKCKVSNKALPAPIEKTISKAKGQPREPQVYTLPPSREEMTKNQVSLTCLVKGFYPSDIAVEWESNGGGGSGGGGSEVQLVESGGGLVQPGGSLRLSCAASGFTFSRYWMSWVRQAPGKCLEWVANIKQDGSEKYYVDSVKGRFTISRDNAKNSLYLQMNSLRAEDTAVYYCAREGGWFGELAFDYWGQGTLVTVSSGGGGSGGGGSGGGGSGGGGSEIVLTQSPGTLSLSPGERATLSCRASQRVSSSYLAWYQQKPGQAPRLLIYDASSRATGIPDRFSGSGSGTDFTLTISRLEPEDFAVYYCQQYGSLPWTFGCGTKVEIKGGGGSGGGGSGQPENNYKTTPPVLDSDGSFFLYSKLTVDKSRWQQGNVFSCSVMHEALHAHYTQKSLSLSPGK

SEQ ID NO: 95 - protein, 707 aa, synthetic construct
  REGION 1..707: note = BiS2-PD-1- OX40 HC -4P
DIQMTQSPSSLSASVGDRVTITCRASQDISNYLNWYQQKPGKAPKLLIYYTSKLHSGVPSRFSGSGSGTDYTLTISSLQPEDFATYYCQQGSALPWTFGCGTKVEIKGGGGSGGGGSGGGGSGGGGSQVQLQESGPGLVKPSQTLSLTCAVYGGSFSSGYWNWIRKHPGKCLEYIGYISYNGITYHNPSLKSRITINRDTSKNQYSLQLNSVTPEDTAVYYCARYKYDYDGGHAMDYWGQGTLVTVSSGGGGSGGGGSEVQLVESGGGLVQPGGSLRLSCAASGFTFSDYGMHWVRQAPGKGLEWVAYISSGSYTIYSADSVKGRFTISRDNAKNSLYLQMNSLRAEDTAVYYCARRAPNSFYEYYFDYWGQGTTVTVSSASTKGPSVFPLAPCSRSTSESTAALGCLVKDYFPEPVTVSWNSGALTSGVHTFPAVLQSSGLYSLSSVVTVPSSSLGTKTYTCNVDHKPSNTKVDKRVESKYGPPCPPCPAPEFLGGPSVFLFPPKPKDTLMISRTPEVTCVVVDVSQEDPEVQFNWYVDGVEVHNAKTKPREEQFNSTYRVVSVLTVLHQDWLNGKEYKCKVSNKGLPSSIEKTISKAKGQPREPQVYTLPPSQEEMTKNQVSLTCLVKGFYPSDIAVEWESNGQPENNYKTTPPVLDSDGSFFLYSRLTVDKSRWQEGNVFSCSVMHEALHNHYTQKSLSLSLGK

SEQ ID NO: 96 - protein, 707 aa, synthetic construct
  REGION 1..707: note = BiS3-OX40 HC-4P-PD-1
EVQLVESGGGLVQPGGSLRLSCAASGFTFSDYGMHWVRQAPGKGLEWVAYISSGSYTIYSADSVKGRFTISRDNAKNSLYLQMNSLRAEDTAVYYCARRAPNSFYEYYFDYWGQGTTVTVSSASTKGPSVFPLAPCSRSTSESTAALGCLVKDYFPEPVTVSWNSGALTSGVHTFPAVLQSSGLYSLSSVVTVPSSSLGTKTYTCNVDHKPSNTKVDKRVESKYGPPCPPCPAPEFLGGPSVFLFPPKPKDTLMISRTPEVTCVVVDVSQEDPEVQFNWYVDGVEVHNAKTKPREEQFNSTYRVVSVLTVLHQDWLNGKEYKCKVSNKGLPSSIEKTISKAKGQPREPQVYTLPPSQEEMTKNQVSLTCLVKGFYPSDIAVEWESNGQPENNYKTTPPVLDSDGSFFLYSRLTVDKSRWQEGNVFSCSVMHEALHNHYTQKSLSLSLGKGGGGSGGGGSDIQMTQSPSSLSASVGDRVTITCRASQDISNYLNWYQQKPGKAPKLLIYYTSKLHSGVPSRFSGSGSGTDYTLTISSLQPEDFATYYCQQGSALPWTFGCGTKVEIKGGGGSGGGGSGGGGSGGGGSQVQLQESGPGLVKPSQTLSLTCAVYGGSFSSGYWNWIRKHPGKCLEYIGYISYNGITYHNPSLKSRITINRDTSKNQYSLQLNSVTPEDTAVYYCARYKYDYDGGHAMDYWGQGTLVTVSS

SEQ ID NO: 97 - protein, 219 aa, synthetic construct; identical to SEQ ID NO: 2
  REGION 1..219: note = PD1 LCv kappa